European Patent Specification EP 3 415 638 B1, published October 8, 2025. Title: Nucleic Acid Amplification Controls and Kits and Methods of Use Thereof. Applicant: IDEXX Laboratories. The sequence listing filed with the application follows.

SEQUENCE LISTING (22 sequences)

SEQ ID NO: 1 - RNA, 80 nt, Unknown
  RNA Internal Positive Control
ggcuccaggauugcucuucagguaucuccccucuuugagaagggccacaucccuacuucuaguuucagcuggaaaggcuu

SEQ ID NO: 2 - DNA, 80 bp, Unknown
  DNA Internal Positive Control
agacaagctggtggcctgaaagaatctcccctctttgagaagggccacatccctacttctagtttcagctggaaaggctt

SEQ ID NO: 3 - DNA, 22 bp, Unknown
  RNA Internal Positive Control forward primer
gctccaggattgctcttcaggt

SEQ ID NO: 4 - DNA, 21 bp, Unknown
  DNA Internal Positive Control forward primer
gacaagctggtggcctgaaag

SEQ ID NO: 5 - DNA, 26 bp, Unknown
  Conserved hydrolysis probe
ctcccctctttgagaagggccacatc

SEQ ID NO: 6 - DNA, 27 bp, Unknown
  Conserved reverse primer
agcctttccagctgaaactagaagtag

SEQ ID NO: 7 - DNA, 28 bp, Mycoplasma gallisepticum
ctgggttgattgttgtttctttactctt

SEQ ID NO: 8 - DNA, 30 bp, Mycoplasma gallisepticum
cttagcgatcggaatcccaatccctaaacc

SEQ ID NO: 9 - DNA, 26 bp, Mycoplasma gallisepticum
acgttcttggatcatcattctttctt

SEQ ID NO: 10 - DNA, 20 bp, Unknown
  T7 phage promoter
taatacgactcactataggg

SEQ ID NO: 11 - DNA, 140 bp, Unknown
  Artificial Signature Sequence
ctccacttcaggtatcactcagtttgaactgcaagacaagctgaaagaatctcgagaagggccacttctagtttcaggcttgggcacagcagatgaaaataaagaaagaaaggaccaggccaaggctacaggccaaagat

SEQ ID NO: 12 - DNA, 24 bp, Unknown
  Primer for artificial Signature Sequence
caagctgaaagaatctcgagaagg

SEQ ID NO: 13 - DNA, 27 bp, Unknown
  Primer for artificial Signature Sequence
ctggtcctttctttctttattttcatc

SEQ ID NO: 14 - DNA, 28 bp, Unknown
  Probe for artificial Signature Sequence
ccacttctagtttcaggcttgggcacag

SEQ ID NO: 15 - DNA, 26 bp, Unknown
  Artificial primer for eukaryotic 18S DNA
gattaagccatgcatgtctaagtacg

SEQ ID NO: 16 - DNA, 28 bp, Unknown
  Artificial primer for eukaryotic 18S DNA
caaaggaaccataactgatttaatgagc

SEQ ID NO: 17 - DNA, 24 bp, Unknown
  Artificial probe for eukaryotic 18S DNA
cacggccggtacagtgaaactgcg

SEQ ID NO: 18 - DNA, 20 bp, Unknown
  Artificial primer for bacterial 16S ribosomal DNA
ggatgatcagccacactgga

SEQ ID NO: 19 - DNA, 21 bp, Unknown
  Artificial primer for bacterial 16S ribosomal DNA
ccaatattcctcactgctgcc

SEQ ID NO: 20 - DNA, 26 bp, Unknown
  Artificial probe for bacterial 16S ribosomal DNA
cccgtaggagtctggaccgtgtctca

SEQ ID NO: 21 - RNA, 183 nt, Bos taurus
gaaugaaguggaccuaguuguucauucgcugaaggaccugcccacggugcuuccuccuggcuucaccauuggagcugucugcaagcgggagagccccuaugaugcuguugucuuucacccaaaauuuguugggaagacucuagaaaccuugccagagaagagugugguaggaacuagcucccu

SEQ ID NO: 22 - RNA, 78 nt, Bos taurus
gaaugaaguggaccuaguuguucauuccgugcuuccuccuggcuucaccuagaagagugugguaggaacuagcucccu